European Patent Application EP 4 800 112 A1, published September 2, 2026. Title: CRISPR-Cas-Loaded Bacteriophages and Uses Thereof. Applicant: CHUNG ANG University Industry Academic Cooperation Foundation. The sequence listing filed with the application follows.

SEQUENCE LISTING (22 sequences)

SEQ ID NO: 1 - DNA, 58 bp, synthetic construct
  source 1..58: mol_type = other DNA
gcctacaatccccggtatacgaattccgagctcaaaaaaaaggcggtgatgtaaacac

SEQ ID NO: 2 - DNA, 59 bp, synthetic construct
  source 1..59: mol_type = other DNA
gcaaaaggggatgataagtttgggatccgtataccgtgtaggctggattccggggatcc

SEQ ID NO: 3 - DNA, 59 bp, synthetic construct
  source 1..59: mol_type = other DNA
accgccttttttttgagctcggaattcgtataccggggattgtaggctggagctgcttc

SEQ ID NO: 4 - DNA, 59 bp, synthetic construct
  source 1..59: mol_type = other DNA
cccggaatccagcctacacggtatacggatcccaaacttatcatccccttttgcttatg

SEQ ID NO: 5 - DNA, 26 bp, synthetic construct
  source 1..26: mol_type = other DNA
atcggggaaggattccacgctgcagc

SEQ ID NO: 6 - DNA, 26 bp, synthetic construct
  source 1..26: mol_type = other DNA
gacaagctccggtcttaatcgacagc

SEQ ID NO: 7 - DNA, 17 bp, synthetic construct
  source 1..17: mol_type = other DNA
actcgtcgcgaaccgct

SEQ ID NO: 8 - DNA, 24 bp, synthetic construct
  source 1..24: mol_type = other DNA
tttgtaggctgtaactgcgggatc

SEQ ID NO: 9 - DNA, 24 bp, synthetic construct
  source 1..24: mol_type = other DNA
aaacatccgacattgacgccctag

SEQ ID NO: 10 - RNA, 20 nt, synthetic construct
  source 1..20: mol_type = other RNA
taggctgtaactgcgggatc

SEQ ID NO: 11 - RNA, 16 nt, synthetic construct
  source 1..16: mol_type = other RNA
taggctgtaactgcgg

SEQ ID NO: 12 - RNA, 15 nt, synthetic construct
  source 1..15: mol_type = other RNA
taggctgtaactgcg

SEQ ID NO: 13 - DNA, 24 bp, synthetic construct
  source 1..24: mol_type = other DNA
tttgtaggctgaaactgcgggatc

SEQ ID NO: 14 - DNA, 24 bp, synthetic construct
  source 1..24: mol_type = other DNA
aaacatccgactttgacgccctag

SEQ ID NO: 15 - DNA, 20 bp, synthetic construct
  source 1..20: mol_type = other DNA
cttgaacatatatctcaggg

SEQ ID NO: 16 - DNA, 20 bp, synthetic construct
  source 1..20: mol_type = other DNA
gaacttgtatatagagtccc

SEQ ID NO: 17 - RNA, 16 nt, synthetic construct
  source 1..16: mol_type = other RNA
aacatatatctcaggg

SEQ ID NO: 18 - DNA, 20 bp, synthetic construct
  source 1..20: mol_type = other DNA
cttgagcatatatctcaggg

SEQ ID NO: 19 - DNA, 20 bp, synthetic construct
  source 1..20: mol_type = other DNA
gaactcgtatatagagtccc

SEQ ID NO: 20 - DNA, 20 bp, synthetic construct
  source 1..20: mol_type = other DNA
tttgctgtggatatacgagg

SEQ ID NO: 21 - DNA, 20 bp, synthetic construct
  source 1..20: mol_type = other DNA
aaacgacacctatatgctcc

SEQ ID NO: 22 - RNA, 16 nt, synthetic construct
  source 1..16: mol_type = other RNA
ctgtggatatacgagg